European Patent Application EP 4 741 491 A1, published May 13, 2026. Title: 产L-缬氨酸工程菌及构建方法与应用. Applicant: 黑龙江伊品生物科技有限公司. Application CN. The sequence listing filed with the application follows.

SEQUENCE LISTING (73 sequences)

SEQ ID NO: 1 - DNA, 2579 bp, Artificial sequence
  source 1..2579: mol_type = other DNA
gagtgatgagcggttgaaggatatcgggttacgcagggaggatgtggagtgaggggggatatagatttatatataataaaacgtttttatgtttttaaattaagttataaaaattttcccgagacaattcatcaataggtatggagtgtacaggaatatcttcttcactaacctctttaaactcatgtcgataacggtcaaaaaacgcacagtgattacttgtgttttttgactgactttacaactctcattattcgctattgtgcagtttctctaattgttttataccctggaaagttaaatgtcagctactgaatactttttgattgtttgagatttattttcatttgaaattataaaatcaggtgataaatgagttgtgattaatagatggttgatatcatttttatctaaaattgatttatagtatcgacctgaaaaaatagttgttgccgcctgagtaactatacaatattctgaaaggttttctttcaaattagaaatgttgtggggttttgtttttgtatcttttatctctaaggagcttgctttgggtcaatcagaatacatttcatgggtaaaatgtacttcctggctaagtaactttgtgaatcttagagggttgagacaaccggatggccgtcctctttatgaatatcatgcaaccaatgatgaatatacccaattaacgcagctactccgtgcagtcggtcaatcacaatctaatatatgtaatagggactttgctgcctgttttttgacaattaatcatccggctcgtataatgtgtggaattgtgagcggataacaatttcacacaggaaacagaccgtgcaaaaaacgcaagagattcattcaagcctggaggtgtcgccatccaaggcagccctggaaccagatgataaaggttatcggcgctacgaaatcgcgcaaggtctaaaaacctcccttgctgcaggtttgggcatgtacccgattggtattgcgtttggtctcttggttattcaatacggctacgaatggtgggcagccccactgttttccggcctgattttcgcgggctccaccgaaatgctggtcatcgccctcgttgtgggcgcagcgcccctgggcgccatcgcgctcaccacattgctggtgaacttccgccacgtattctatgcgttttcattcccgctgcatgtggtcaaaaaccccattgcccgtttctattcggttttcgcgcttatcgacgaagcctacgcagtcactgcggccaggcccgcaggctggtcggcgtggcgacttatctcaatgcaaatagcgtttcactcctactgggtattcggcggtctcaccggagtggcgatcgcagagttgattccttttgaaattaagggcctcgagttcgccctttgctctctctttgtcacgctgactttggattcctgccgaacgaaaaagcagatcccttctctgctgctcgcaggtttgagcttcaccattgctcttgtggtaattccaggtcaggccctatttgcggcgctgctgatcttcttgggtctgttgaccatccggtacttcttcttgggaaaggctgctaaatgacaactgatttctcctgtattctccttgttgtcgcagtatgtgcagtcattacttttgcgctccgggcggttccgttcttaatccttaagcccctacgtgaatcacaatttgtgggcaaaatggcgatgtggatgccagcaggaatccttgccattttgaccgcatcaacgtttcgcagcaatgcgatagatctgaagactctaacctttggtctcattgccgttgcgattacagtggtggcgcatcttcttggcggtcgacgcaccttgttgagcgttggcgctggcaccatcgtttttgttggactggtgaatcttttctaactaaaagcactacctgtgaagggatgtcaggacgttacagttacagcaaatgaaacttatcggattcgcaccggaagagaacaaatcagcatcggaaggtttgctctaaatggaaagcgtgcaagctgggtttgtcatccagatgaaacatttattggtgtaccaaaagtcatttctacactaccggatattcaaagcattgatgtaacgcgttacacgtgctgacaaaacagcattacagccagcaggaagtactgcgttggatcgatgtctgttcagggactcaacctaatgcaaaggatcccgcatttcttaaagtcagggcgcatatcttccagcgtaatacctagggaatatgggcttgtgttgataaagattgcagattaaagcacggtacaccgctcgacaaaggctggccctttggctatgtgtatgtgaaccagcgacaaaattgtgactgtggaagccctgtatacgaagttgcattctgtaatgattgtaatgagcctcatcttctggcacgggacaaaaagggcaaactagtccagtgggaaaataaaggtggcgatgaattctctttgcaggatgaagtacctgttgaacatgacgctacagaagaaaaagtcgaaaaagagaacagttttcagcctccgttgattattgccgcag

SEQ ID NO: 2 - protein, 251 aa, Corynebacterium glutamicum
VQKTQEIHSSLEVSPSKAALEPDDKGYRRYEIAQGLKTSLAAGLGMYPIGIAFGLLVIQYGYEWWAAPLFSGLIFAGSTEMLVIALVVGAAPLGAIALTTLLVNFRHVFYAFSFPLHVVKNPIARFYSVFALIDEAYAVTAARPAGWSAWRLISMQIAFHSYWVFGGLTGVAIAELIPFEIKGLEFALCSLFVTLTLDSCRTKKQIPSLLLAGLSFTIALVVIPGQALFAALLIFLGLLTIRYFFLGKAAK

SEQ ID NO: 3 - protein, 108 aa, Corynebacterium glutamicum
MTTDFSCILLVVAVCAVITFALRAVPFLILKPLRESQFVGKMAMWMPAGILAILTASTFRSNAIDLKTLTFGLIAVAITVVAHLLGGRRTLLSVGAGTIVFVGLVNLF

SEQ ID NO: 4 - DNA, 4732 bp, Artificial sequence
  source 1..4732: mol_type = other DNA
tgaatggactgctatgcgcagcctctgtagaggctaagcctcgactacaaaaaaataagagtacgcgttgccaattctattggtcagaaaagcatccagatgagcttagggtgatagtatctcttccggacgaagtttcctttcctgtaacaagcgagccgtcaactacgcgctttgaacttgccatttgtgaagatggtgaggaagtctctggccttgggccagcctatgcttctctggaaaacagacaggcaacagttcgattacgtaaaagcgaagtgagatttggcaggcaaaatccatcggcaggtttgtcgttagtggctcgtgctggagggatgattgttgggagcattaaacttgatgacagtgaaattgccattggtgaggtgccgttaaccttcatcgttgatgcagatcaatggctgttacagggacaggcttcttgcagtgtgcgaagcagcgatgttctgattgtgctccctcgggataatagcaatgttgctggttttgatggccaatcgagggcagtaaacgtattaggactaaaagcactacctgtgaagggatgtcaggacgttacagttacagcaaatgaaacttatcggattcgcaccggaagagaacaaatcagcatcggaaggtttgctctaaatggaaagcgtgcaagctgggtttgtcatccagatgaaacatttattggtgtaccaaaagtcatttctacactaccggatattcaaagcattgatgtaacgcgttacacgtgctgacaaaacagcattacagccagcaggaagtactgcgttgttaacgtctgcttaatacactgtggccgttttgcaaaaactggcttcttgagcggcgcatgcgttcaatccgttcctctgctaagcggtcagccgctaaatatgcaggaatgccgtcacgctgagaaatctcaagtacacgctcgatattgccgtaaatgccttcaacttttttcaatgcacgttctgcattatagccgtaaagctcatctgccacgttgatgacaccgcccgcgttaatcacgtaatccggtgcataaacgatgcccatttcgtgaatttgatcaccatggcgtgtctcttttaattggttgttagccgcacctgcgatcactttcgccttcagctgtttaatggtgtcgtcgttaatagtcgcaccaagggcacacggcgcataaatatcgcagtcttgtgaataaatgtcatcaggatctaccgcacgggcgccaaaatcttcaactgcacgctgtacagattgtttgttgatatccgtaacgattaagtttgctccttcttcatgcaggtggcggcaaaggttataggctacgttcccaacaccctgtacagcaatggtttttccttcaagagagtcggttccgaaagcagctttagctgctgccttcattcctctgtacaccccgtacgctgtgactggggacggatttccagaagagccgaaagcaggagaaatccctgtgacatagtctgtctcatcatgaatgatatccatatcctcgaccgttgtgcccacatcttcagccgtgatgtatctgccattcagtccttgaatatagcggccaaacgcgcggaacatttcctcatttttgtctttgcgcggatcgccgataatgactgtttttccgccgccaaggtttaagcctgccgccgcgttcttataggtcatgcctcttgccaatctgagcgcatcttcaattgccgcttcttcattttcatatgtccacattctcgttccgccaagcgccggaccaagcgttgtatcatgaatggcgataatcgcttttaatccagattgttcatcctggcagaataccaattgttcgtaatcgtatttctccatatatttaaaaagttccatggtctgtttcctgtgtgaaattgttatccgctcacaattccacacattatacgagccggatgattaattgtcaattaaccccccagtttcgatttatcgcgcaccgcgcctttgtcggcgctggttgccaggctggcataagcacgcagggcaaaggagacctgacgttcacgatttttcggcgtccaggctttgtcacctcgagcgtcctgcgcttcacgacgcgccgccagttcggcatcgcttacctgtaactgaatgccacggttcgggatgtcgatagcgatcaggtcaccatcttcaatcaggccaatgctgccgccgcttgccgcttccggtgagacgtggccgatggaaagaccagaggtgccaccagagaaacgaccgtcggtgatcagcgcacaggctttgccgagacccattgatttcaggaagctggttgggtagagcatttcctgcatccccggaccgcctttcgggccttcatagcgaattactaccacatctccggcgacaactttaccgccgagaatcgcttctaccgcatcgtcctggctttcgtacactttcgccgggccggtgaatttgaggatgctgtcatcgacgcctgccgttttcacgatgcagccgttttccgcaaagttaccgtagagcaccgccaggccgccgtctttgctgtaggcgtgttccagcgagcggatacagccattggcgcgatcgtcgtccagcgtatcccaacggcaatcttgcgagaatgcctgtgtggtacgaatgcctgcaggacctgcgcggaacatattttttaccgcgtcatcctgggtcagcataacgtcgtattgttccagcgtttgcggcaacgtcaggccaagtacgtttttcacatcacggttcagtaaccccgcgcgatccagttcgccgagaataccgataacaccaccagcacggtgaacatcttccatatggtatttctgggtgctcggcgcaactttacacagctgtggaaccttgcgggaaagcttatcgatatcactcatggtgaagtcgatttccgcttcctgcgccgccgccagcaggtgaagtacggtgttagtcgatccacccatcgcgatatccagcgtcatggcgttttcaaacgccgccttactggcgatattacgcggcagtgcactttcgtcgttttgctcgtaataacgtttggtcaattcaacaatgcgtttaccagcattaaggaacagctgcttacggtcggcgtgggttgccagcagcgagccgttgcccggctgcgacaggcccagcgcttcggtcaggcagttcattgagttagcggtaaacatcccggagcaggaaccgcaggtcggacacgcggaacgttcaacctgatcgctctgggagtcagatactttcgggtctgcgccctggatcatcgcatcaaccagatcgagcttgatgatctgatcggaaagtttggttttcccggcctccatcgggccgccggaaacaaagatcaccggaatattcaggcgcagggaagccatcagcatccccggggtgattttgtcgcagttagagatgcagaccatggcgtcggcgcagtgggcgttgaccatatactcaacggaatcagcgatcagttcgcgagatggcagtgaataaagcatccccccgtggcccatggcaatcccatcatccaccgcaatggtgttgaactctttggcaacgccgccagccgcttcaatttgttcggcgaccagtttaccgagatcgcgcagatggacgtgacccggtacaaattgggtgaacgagttcacaaccgcgataatcggcttaccgaaatcggcgtcggtcattccggtggcgcgccacagcgcacgagcacccgccatattacgaccatgagtggtggtggcggaacggtacttaggcatactttatttactcccagtgtctgtctcgtaaatgggacggtgcgtgccgtcccattttttgtatttcaacggatgtgctggtggaggtgatcgcctcctgatgatgagccgctcccgatgtggtgtcgggagcggtattttctataaaacttaccgcttatttgagatattcatcgaaaatgtcgagtaattcttgatgtatacacggccattcctgacctaaattgacggtacacaagccaatatcgaagccattaattttataacgatgtttcactgcggtatctacgtggggatatattaataacccccctatgttttcgccattttcaggctttaacgaccataagtaattcatcagttgataaagattttgcgaatgaaatttttctgttcccattcgtcgtgaaaaaatgctcttatagtatttggcgtcaacgataagtattttttctgatgagcgaatggtgatgtcagtttccattcgaggtaacaaattaagtgactgatccgatatactcgatgcatcccattttaaataagagcgggttgtgtttgcagacgttaattcacgacggcaaaattcataaagaaacttttgataaagtaatgacatctctttttcgtttctttcaaaatcatagaaacggtagtgtcctttgttttgacctggaatagaattattgacgatgaatttgcagacactgataacgaatttataataacgcgtattttttccgccattcagatagctgaaatgctgcggagttaaatgaagagtgctaatgcccggtaattttctataaagtgaacgagcttcatctctgatagttgaatttaacttttcatgcttaattaatatggctaatgtgctttttataattcggttagccagcgtgtcttca

SEQ ID NO: 5 - protein, 616 aa, Escherichia coli
MPKYRSATTTHGRNMAGARALWRATGMTDADFGKPIIAVVNSFTQFVPGHVHLRDLGKLVAEQIEAAGGVAKEFNTIAVDDGIAMGHGGMLYSLPSRELIADSVEYMVNAHCADAMVCISNCDKITPGMLMASLRLNIPVIFVSGGPMEAGKTKLSDQIIKLDLVDAMIQGADPKVSDSQSDQVERSACPTCGSCSGMFTANSMNCLTEALGLSQPGNGSLLATHADRKQLFLNAGKRIVELTKRYYEQNDESALPRNIASKAAFENAMTLDIAMGGSTNTVLHLLAAAQEAEIDFTMSDIDKLSRKVPQLCKVAPSTQKYHMEDVHRAGGVIGILGELDRAGLLNRDVKNVLGLTLPQTLEQYDVMLTQDDAVKNMFRAGPAGIRTTQAFSQDCRWDTLDDDRANGCIRSLEHAYSKDGGLAVLYGNFAENGCIVKTAGVDDSILKFTGPAKVYESQDDAVEAILGGKVVAGDVVVIRYEGPKGGPGMQEMLYPTSFLKSMGLGKACALITDGRFSGGTSGLSIGHVSPEAASGGSIGLIEDGDLIAIDIPNRGIQLQVSDAELAARREAQDARGDKAWTPKNRERQVSFALRAYASLATSADKGAVRDKSKLGG

SEQ ID NO: 6 - protein, 364 aa, Bacillus subtilis
MELFKYMEKYDYEQLVFCQDEQSGLKAIIAIHDTTLGPALGGTRMWTYENEEAAIEDALRLARGMTYKNAAAGLNLGGGKTVIIGDPRKDKNEEMFRAFGRYIQGLNGRYITAEDVGTTVEDMDIIHDETDYVTGISPAFGSSGNPSPVTAYGVYRGMKAAAKAAFGTDSLEGKTIAVQGVGNVAYNLCRHLHEEGANLIVTDINKQSVQRAVEDFGARAVDPDDIYSQDCDIYAPCALGATINDDTIKQLKAKVIAGAANNQLKETRHGDQIHEMGIVYAPDYVINAGGVINVADELYGYNAERALKKVEGIYGNIERVLEISQRDGIPAYLAADRLAEERIERMRRSRSQFLQNGHSVLSRR

SEQ ID NO: 7 - DNA, 2108 bp, Artificial sequence
  source 1..2108: mol_type = other DNA
ccaatctggtgaagagcaagtcaaaaacagagcaggctcaactggcgcggtatgctttcaacaaccaatggtgggatcttagcgttcaggcaacgatcgccgggaagctgtgggatcatctggaagagcgattcccgctggcttacaacgatcttttcaaacgctacaccagcggtaaggagatcccgcaaagctatgcgatggcgattgctcgtcaggagagcgcctggaatccgaaagtgaaatcaccggtaggggccagcggcttgatgcagattatgcctggtacagcgacccatacggtgaagatgttctctattcccggttatagcagtcctgggcaattgctggatccggaaacgaatatcaacattggcaccagttacctgcaatatgtttatcagcagtttggcaataatcgtattttctcctcagcagcttataacgccggaccagggcgggtgcgaacctggcttggcaacagcgccgggcgtatcgacgcagtggcatttgtcgagagtattccattctccgagacgcgcggttatgtgaagaacgtgctggcttatgacgcttactaccgctatttcatgggggataaaccgacgttgatgagcgccacggaatggggacgtcgttactgatccgcacgtttatgatatgctatcgtactctttagcgagtacaaccgggggaggcattttgcttcccccgctaacaatggcgacatattatggcccaacaatcaccctattcagcattgacaattaatcatccggctcgtataatgtgtggaattgtgagcggataacaatttcacacaggaaacagaccatgcgccggatattatcagtcttactcgaaaatgaatcagacgcgttattccgcgtgattggccttttttcccagcgtggctacaacattgaaagcctgaccgttgcgccaaccgacgatccgacattatcgcgtatgaccatccagaccgtgggcgatgaaaaagtacttgagcagatcgaaaagcaattacacaaactggtcgatgtcttgcgcgtgagtgagttggggcagggcgcgcatgttgagcgggaaatcatgctggtgaaaattcaggccagcggttacgggcgtgacgaagtgaaacgtaatacggaaatattccgtgggcaaattatcgatgtcacaccctcgctttataccgttcaattagcaggcaccagcggtaagcttgatgcatttttagcatcgattcgcgatgtggcgaaaattgtggaggttgctcgctctggtgtggtcggactttcgcgcggcgataaaataatgcgttgatttggtaggcatgataagacgcggcagcgtcgcatcaggcgcttaatacacggcattatgaaacggactcagcgccaggatcaccgcctggtgatagacgctggcgcgagtgagtttcccggcggtaaacacgccgatcgccccttccttacgaccaatctcatcaataccggtataacgcgacatcacgggaccaagcgcctcaccttcacgcactttttccagaatcaccgcaggcaacggcaaagtagccgaacgcgcctcgccgcgctggctggcgttttcaatcaccacccaactgaaagtgctgtcaccatcgatgccagcttcaatcgccacccaaaaatcagcctctggaagtaaacggcgggcattggctacccgatttcgtgcgccagcgcgcgtttcctcactgccaaagggctgttccggtacaccgctctcgacggcaacggatgcaatatggcaggatccttcgccgaagatctcgtgaaatgcctgcagaatggcctgaattttagcgggattggtggtcgcacagacaacttggtgcataatcagcattactcagaaaattaacgttacagcagtatacggaaaaaaagcatgttacaggtatacctagtccgccacggtgaaacgcagtggaacgccgagcgacgtattcagggccagtctgacagcccgctgaccgccaaaggtgagcaacaggcgatgcaggtggcaacccgtgccaaagagcttggcattacgcatatcatcagtagcgatttaggacgcac

SEQ ID NO: 8 - protein, 163 aa, Artificial sequence
MRRILSVLLENESDALFRVIGLFSQRGYNIESLTVAPTDDPTLSRMTIQTVGDEKVLEQIEKQLHKLVDVLRVSELGQGAHVEREIMLVKIQASGYGRDEVKRNTEIFRGQIIDVTPSLYTVQLAGTSGKLDAFLASIRDVAKIVEVARSGVVGLSRGDKIMR

SEQ ID NO: 9 - DNA, 4524 bp, Artificial sequence
  source 1..4524: mol_type = other DNA
cggtaataatccacagcaggtatttgcgcagcccgagtttgtcagaaagcagaccaaacagcggttggaataatagcgagaacagagaaatagcggcaaaaataatacccgtatcacttttgctgatatggttgatgtcatgtagccaaatcgggaaaaacgggaagtaggctcccatgataaaaaagtaaaagaaaaagaataaaccgaacatccaaaagtttgtgttttttaaatagtacataatggatttccttacgcgaaatacgggcagacatggcctgcccggttattattatttttgacaccagaccaactggtaatggtagcgaccggcgctcagctggaattccgccgatactgacgggctccaggagtcgtcgccaccaatccccatatggaaaccgtcgatattcagccatgtgccttcttccgcgtgcagcagatggcgatggctggtttccatcagttgctgttgactgtagcggctgatgttgaactggaagtcgccgcgccactggtgtgggccataattcaattcgcgcgtcccgcagcgcagaccgttttcgctcgggaagacgtacggggtatacatgtctgacaatggcagatcccagcggtcaaaacaggcggcagtaaggcggtcgggatagttttcttgcggccctaatccgagccagtttacccgctctgctacctgttacgcgaacgcgaagtccgactctaagatgtcacggaggttcaagttacctttagccggaagtgctggcattttgtccaattgagactcgtgcaactggtcagcgaactggtcgtagaaatcagccagtacatcacaagactcatatgtgtcaaccatagtttcgcgcactgctttgaacaggttcgcagcgtcagccggaatggtaccgaaggagtcgtgaatcagtgcaaaagattcgattccgtacttctcgtgtgcccacactacagtcttacgaaggtggctaccgtcttggctgtgtacaaagttaggagcgataccagactcctgtttgtgtgcatcaatctcgctatctttgttggtgttaatggtaggctgtaagcggaactgaccgaggaacatcaggttcaagcgcgtctgaataggcttcttgtattcctgccacacagggaaaccatcaggagttacccaatgcacagcgcaacgcttgcgaagaatctctccagtcttcttatctttgacctcagcagccagcagcttagcagcagacttaagccagttcattgcttcaaccgcagctaccaccgtcacgctcacagattcccaaatcagcttagccatgtatccagcagcctgattcggctgagtgaacatcagacccttgccggaatcaatagctggctgaatggtatcttccagcacttgttgacggaagccgaactctttggacccgtaagccagcgtcatgactgaacgcttagtcacactgcgagtaacaccgtaagccagccattgaccagccagtgccttagtgcccagcttgactttctcagagatttcaccagtgttctcatcggtcacggtaactacttcgttatcggtcccattgattgcgtctgcttgtagaatctcgttgactttcttagcaacaatcccgtagatgtcctgaacggtttcactaggaagcaagttaaccgcgcgaccacctacctcatctcggagcatcgcggagaagtgctggatgccagagcaagacccgtcaaacgccagcggaagggagcagttatagctcaggccgtggtgctgtaccccagcgtactcaaagcagaacgcaaggaagcagaacggagaatcttgctcagcccaccaagtgttctccagtggagacttagcgcaagccatgatgttctcgtggttttcctcaatgaacttgatgcgctcagggaacggaaccttatcgacacccgcacagtttgcaccgtggattttcagccagtagtaaccttccttaccgattggtttacctttcgccagcgtaagcagtcctttggtcatatcgttaccttgcgggttgaacattgacacagcgtaaacacgaccgcgccagtccatgttgtaagggaaccagatggccttatggttagcaaacttattggcttgctcaagcatgaactcaaggctgatacggcgagacttgcgagccttgtccttgcggtacacagcagcggcagcacgtttccacgcggtgagagcctcaggattcatgtcgatgtcttccggtttcatcgggagttcttcacgctcaatcgcagggatgtcctcgaccggacaatgcttccacttggtgattacgttggcgaccgctaggactttcttgttgattttccatgcggtgttttgcgcaatgttaatcgctttgtacacctcaggcatgtaaacgtcttcgtagcgcatcagtgctttcttactgtgagtacgcaccagcgccagaggacgacgaccgttagcccaatagccaccaccagtaatgccagtccacggcttaggaggaactacgcaaggttggaacatcggagagatgccagccagcgcacctgcacgggttgcgatagcctcagcgtattcaggtgcgagttcgatagtctcagagtcttgacctactacgccagcattttggcggtgtaagctaaccattccggttgactcaatgagcatctcgatgcagcgtactcctacatgaatagagtcttccttatgccacgaagaccacgcctcgccaccgagtagacccttagagagcatgtcagcctcgacaacttgcataaatgctttcttgtagacgtgccctacgcgcttgttgagttgttcctcaacgtttttcttgaagtgcttagcttcaaggtcacggatacgaccgaagcgagcctcgtcctcaatggcccgaccgattgcgcttgctacagcctgaacggttgtattgtcagcactggttaggcaagccagagtggtcttaatggtgatgtacgctacggcttccggcttgatttcttgcaggaactggaaggctgtcgggcgcttgccgcgcttagctttcacttcctcaaaccagtcgttgatgcgtgcaatcatcttagggagtagggtagtgatgagaggcttggcggcagcgttatccgcaacctcaccagctttaagttgacgctcaaacatcttgcggaagcgtgcttcacccatctcgtaagactcatgctcaagggccaactgttcgcgagctaaacgctcaccgtaatggtcagccagagtgttgaacgggatagcagccagttcgatgtcagagaagtcgttcttagcgatgttaatcgtgttcatggtgtagggccttctgtagttagaggacagttttaataagtaacaatcaccgcgataaacgtaaccaatttttagcaactaaacaggggaaaacaattacagatttttatctttcgattacgatttttggtttatttcttgatttatgaccgagatcttacttttgttgcgcaattgtacttattgcatttttctcttcgaggaattacccagtttcatcattccattttattttgcgagcgagcgcacacttgtgaattatctccgccgagacagaacttaatgggcccgctaacagcgcgatttgctggtgacccaatgcgaccagatgctccacgcccagtcgcgtaccgtcttcatgggagaaaataatactgttgatgggtgtctggtcagagacatcaagaaataacgccggaacattagtgcaggcagcttccacagcaatggcatcctggtcatccagcggatagttaatgatcagcccactgacgcgttgcgcgagaagattgtgcaccgccgctttacaggcttcgacgccgcttcgttctaccatcgacaccaccacgctggcacccagttgatcggcgcgagatttaatcgccgcgacaatttgcgacggcgcgtgcagggccagactggaggtggcaacgccaatcagcaacgactgtttgcccgccagttgttgtgccacgcggttgggaatgtaattcagctccgccatcgccgcttccactttttcccgcgttttcgcagaaacgtggctggcctggttcaccacgcgggaaacggtctgataagagacaccggcatactctgcgacatcgtataacgttactggtttcacattcaccaccctgaattgactctcttccgggcgctatcatgccataccgcgaaaggttttgcgccattcgatggtgtcaacgtaaatgcatgccgcttcgccttccggccaccagaatagcctgcgattcaaccccttcttcgatctgttttgctacccgttgtagcgccggaagatgcttttccgctgcctgttcaatggtcattgcgctcgccatatacaccagattcagacagccaatcacccgttgttcactgcgcagcggtacggcgatagaggcgatcttctcctcctgatcccagccgcggtagttctgtccgtaacc

SEQ ID NO: 10 - protein, 883 aa, Escherichia coli
MNTINIAKNDFSDIELAAIPFNTLADHYGERLAREQLALEHESYEMGEARFRKMFERQLKAGEVADNAAAKPLITTLLPKMIARINDWFEEVKAKRGKRPTAFQFLQEIKPEAVAYITIKTTLACLTSADNTTVQAVASAIGRAIEDEARFGRIRDLEAKHFKKNVEEQLNKRVGHVYKKAFMQVVEADMLSKGLLGGEAWSSWHKEDSIHVGVRCIEMLIESTGMVSLHRQNAGVVGQDSETIELAPEYAEAIATRAGALAGISPMFQPCVVPPKPWTGITGGGYWANGRRPLALVRTHSKKALMRYEDVYMPEVYKAINIAQNTAWKINKKVLAVANVITKWKHCPVEDIPAIEREELPMKPEDIDMNPEALTAWKRAAAAVYRKDKARKSRRISLEFMLEQANKFANHKAIWFPYNMDWRGRVYAVSMFNPQGNDMTKGLLTLAKGKPIGKEGYYWLKIHGANCAGVDKVPFPERIKFIEENHENIMACAKSPLENTWWAEQDSPFCFLAFCFEYAGVQHHGLSYNCSLPLAFDGSCSGIQHFSAMLRDEVGGRAVNLLPSETVQDIYGIVAKKVNEILQADAINGTDNEVVTVTDENTGEISEKVKLGTKALAGQWLAYGVTRSVTKRSVMTLAYGSKEFGFRQQVLEDTIQPAIDSGKGLMFTQPNQAAGYMAKLIWESVSVTVVAAVEAMNWLKSAAKLLAAEVKDKKTGEILRKRCAVHWVTPDGFPVWQEYKKPIQTRLNLMFLGQFRLQPTINTNKDSEIDAHKQESGIAPNFVHSQDGSHLRKTVVWAHEKYGIESFALIHDSFGTIPADAANLFKAVRETMVDTYESCDVLADFYDQFADQLHESQLDKMPALPAKGNLNLRDILESDFAFA

SEQ ID NO: 11 - DNA, 3189 bp, Artificial sequence
  source 1..3189: mol_type = other DNA
aaatggagggataacagccagcgcagtagtcagtgaatttggtggcaccatctttatgaatggtgataattcagtcgagtcgggtggggcatattcagcgggacttttaagccaggttaatgattctgaaaagatggtaaataacacccgtcttgaaaccacagataaaacgaacattgttacctctggggaaaatgcagtaggtgttcttgcatgttcaagtcctggagagtctcgaacatgtgtcgatgctgtagatgatgaagttagtgattctaacagttacgaagttattagccgtgctgatttaaaaatgaatggtggttccataacaactaatggcattaatagctatggtgcttatgctaatgggaaaaaagcatatattaatttagattatgtggcacttgaaactgtggctgatggaagttatgcagttgctattcgacaaggtaacattgatataaaaaatagttctattacaacaacaggcactaaagcccccattgcaaaaatatacaatggtggagagttatttttttccaatgtcaccgcggtatcaaaacaagataaaggaatatcaattgatgcatcaaatatcgattctcaagccaaaatagcactattaagtgttgaactttcaagtgctttggatagtattgatgttaacaaaactacaacggatgtaagtatccttaatcgaagtattatcacacctggtaataatgttctggttaataatactggaggtgacttaaacataatttcgtccgactctattctaaatggagcgttaacccgcaacagcaatacgtttcatatctgtcatatagccgcgcagtttcttacctacctgctcaatcgcatggctgcgaatcgcttcgttcacatcacgcagttgcccgttatctaccgcgccttccggaatagctttacccaggtcgcccggttgcagctctgccataaacggtttcagcaacggcacacaagcgtaagagaacagatagttaccgtactcagcggtatcagagataaccacgttcatttcgtacagacgcttacgggcgatggtgttggcaatcagcggcagctcgtgcagtgattcataatatgcagactcttcaatgatgccggaatcgaccatggtttcgaacgccagttcaacgcccgctttcaccatcgcaatcatcagtacgcctttatcgaagtactcctgctcgccgattttgccttcatactgcggcgcggtttcaaacgcggttttgccggtctcttcacgccaggtcagcagtttcttatcatcgttggcccagtccgccatcataccggaagagaattcgccggagatgatgtcgtccatatgtttctggaacaggggtgccatgatctctttcagctgttcagaaagcgcataagcacgcagtttcgccgggttagagagacggtccatcatcagggtgatgccgccctgtttcagtgcttcggtgatggtttcccaaccgaactgaatcagtttttctgcgtatgctggatcggtaccttcttccaccagcttgtcgaagcacagcagagagccagcctgcaacataccgcacaggatggtttgctcgcccatcaggtcagatttcacttccgcaacgaaggacgattccagcacacccgcacggtgaccaccggttgcagccgcccaggctttggcaatcgccatgccttcgcctttcggatcgttttccgggtgaacggcaatcagcgtcggtacgccgaacccacgtttgtactcttcacgcacttcggtgcctgggcatttcggcgcaaccatcactacggtgatatctttacggatctgctcgcccacttcgacgatgttgaaaccgtgcgagtagcccagcgccgcgccgtctttcatcagtggctgtacggtgcgcactacatcagagtgctgcttgtccggcgtcaggttaatcaccagatccgcctgtgggatcagttcttcgtaagtacccactttaaaaccattttcggtcgctttacgccaggacgcgcgcttctcggcaatcgcttctttacgcagagcgtaggagatatcgagaccagaatcacgcatgttcaggccctggttcagaccctgtgcgccacagccgacgatgactacttttttaccctgaaggtagctcgcgccatcggcgaattcatcgcggcccataaagcgacatttgcccagctgtgccagctgctggcgcagattcagtgtattgaagtagttagccatggtctgtttcctgtgtgaaattgttatccgctcacaattccacacattatacgagccggatgattaattgtcaaaaacttggcgtaaatggcaacctgaatccagcggccagcgtctggggaatgtgggcgtgcagctgggtgataatggctacaatgacaccgcagtgatggtgggcctgaaatataagttctgatcccgccgttagctaaaaaaccgcgtcgtattcatcgacgcggtacatatgaaatattattttttgccgatagcacgcatggtgtcatcaattgccgtgatcaacagcatttgcgggtctttagcgcaaacctgattcagtttttctaccactttggcgctcagttccggagattgctcaatttttaaatcacggctggcaacgctggcattacccattaccgcaacaatttctgcaacctgtgcgctgtcagtttttgccatttcgttggcttctgcgcaagtaatataggtttctgacggcaaaccgtttttaatattgtagtcctgcgcccaggtcattggtgcgaaaacaaacaggcccgccagtaaagcaaattttttcatcatcattccttatttcattttacccagaattgcaccacccgtaccgccaatcacggcacctttaatcgccccttcgaggccattgccggtcagaacgccagtgacagcaccaacggcggcacccacttttgcacctttacgcgcatttttaccgtcgcggcctttttctgttactgcaccaacaccagcgccaacagctgcacctttcagtacgccattaacaccattgccagtaagtaaaccaacgcctgcgcctagcaatgcacctttcgtggtgcggttcatatccgccatcgctggcgtggagcagaacaatgctgagataagcccgaaggcaa

SEQ ID NO: 12 - protein, 491 aa, Escherichia coli
MANYFNTLNLRQQLAQLGKCRFMGRDEFADGASYLQGKKVVIVGCGAQGLNQGLNMRDSGLDISYALRKEAIAEKRASWRKATENGFKVGTYEELIPQADLVINLTPDKQHSDVVRTVQPLMKDGAALGYSHGFNIVEVGEQIRKDITVVMVAPKCPGTEVREEYKRGFGVPTLIAVHPENDPKGEGMAIAKAWAAATGGHRAGVLESSFVAEVKSDLMGEQTILCGMLQAGSLLCFDKLVEEGTDPAYAEKLIQFGWETITEALKQGGITLMMDRLSNPAKLRAYALSEQLKEIMAPLFQKHMDDIISGEFSSGMMADWANDDKKLLTWREETGKTAFETAPQYEGKIGEQEYFDKGVLMIAMVKAGVELAFETMVDSGIIEESAYYESLHELPLIANTIARKRLYEMNVVISDTAEYGNYLFSYACVPLLKPFMAELQPGDLGKAIPEGAVDNGQLRDVNEAIRSHAIEQVGKKLRGYMTDMKRIAVAG

SEQ ID NO: 13 - DNA, 4713 bp, Artificial sequence
  source 1..4713: mol_type = other DNA
agttcgccctttgctctctctttgtcacgctgactttggattcctgccgaacgaaaaagcagatcccttctctgctgctcgcaggtttgagcttcaccattgctcttgtggtaattccaggtcaggccctatttgcggcgctgctgatcttcttgggtctgttgaccatccggtacttcttcttgggaaaggctgctaaatgacaactgatttctcctgtattctccttgttgtcgcagtatgtgcagtcattacttttgcgctccgggcggttccgttcttaatccttaagcccctacgtgaatcacaatttgtgggcaaaatggcgatgtggatgccagcaggaatccttgccattttgaccgcatcaacgtttcgcagcaatgcgatagatctgaagactctaacctttggtctcattgccgttgcgattacagtggtggcgcatcttcttggcggtcgacgcaccttgttgagcgttggcgctggcaccatcgtttttgttggactggtgaatcttttctaactaaaagcactacctgtgaagggatgtcaggacgttacagttacagcaaatgaaacttatcggattcgcaccggaagagaacaaatcagcatcggaaggtttgctctaaatggaaagcgtgcaagctgggtttgtcatccagatgaaacatttattggtgtaccaaaagtcatttctacactaccggatattcaaagcattgatgtaacgcgttacacgtgctgacaaaacagcattacagccagcaggaagtactgcgttgttaacgtctgcttaatacactgtggccgttttgcaaaaactggcttcttgagcggcgcatgcgttcaatccgttcctctgctaagcggtcagccgctaaatatgcaggaatgccgtcacgctgagaaatctcaagtacacgctcgatattgccgtaaatgccttcaacttttttcaatgcacgttctgcattatagccgtaaagctcatctgccacgttgatgacaccgcccgcgttaatcacgtaatccggtgcataaacgatgcccatttcgtgaatttgatcaccatggcgtgtctcttttaattggttgttagccgcacctgcgatcactttcgccttcagctgtttaatggtgtcgtcgttaatagtcgcaccaagggcacacggcgcataaatatcgcagtcttgtgaataaatgtcatcaggatctaccgcacgggcgccaaaatcttcaactgcacgctgtacagattgtttgttgatatccgtaacgattaagtttgctccttcttcatgcaggtggcggcaaaggttataggctacgttcccaacaccctgtacagcaatggtttttccttcaagagagtcggttccgaaagcagctttagctgctgccttcattcctctgtacaccccgtacgctgtgactggggacggatttccagaagagccgaaagcaggagaaatccctgtgacatagtctgtctcatcatgaatgatatccatatcctcgaccgttgtgcccacatcttcagccgtgatgtatctgccattcagtccttgaatatagcggccaaacgcgcggaacatttcctcatttttgtctttgcgcggatcgccgataatgactgtttttccgccgccaaggtttaagcctgccgccgcgttcttataggtcatgcctcttgccaatctgagcgcatcttcaattgccgcttcttcattttcatatgtccacattctcgttccgccaagcgccggaccaagcgttgtatcatgaatggcgataatcgcttttaatccagattgttcatcctggcagaataccaattgttcgtaatcgtatttctccatatatttaaaaagttccatggtctgtttcctgtgtgaaattgttatccgctcacaattccacacattatacgagccggatgattaattgtcaattaaccccccagtttcgatttatcgcgcaccgcgcctttgtcggcgctggttgccaggctggcataagcacgcagggcaaaggagacctgacgttcacgatttttcggcgtccaggctttgtcacctcgagcgtcctgcgcttcacgacgcgccgccagttcggcatcgcttacctgtaactgaatgccacggttcgggatgtcgatagcgatcaggtcaccatcttcaatcaggccaatgctgccgccgcttgccgcttccggtgagacgtggccgatggaaagaccagaggtgccaccagagaaacgaccgtcggtgatcagcgcacaggctttgccgagacccattgatttcaggaagctggttgggtagagcatttcctgcatccccggaccgcctttcgggccttcatagcgaattactaccacatctccggcgacaactttaccgccgagaatcgcttctaccgcatcgtcctggctttcgtacactttcgccgggccggtgaatttgaggatgctgtcatcgacgcctgccgttttcacgatgcagccgttttccgcaaagttaccgtagagcaccgccaggccgccgtctttgctgtaggcgtgttccagcgagcggatacagccattggcgcgatcgtcgtccagcgtatcccaacggcaatcttgcgagaatgcctgtgtggtacgaatgcctgcaggacctgcgcggaacatattttttaccgcgtcatcctgggtcagcataacgtcgtattgttccagcgtttgcggcaacgtcaggccaagtacgtttttcacatcacggttcagtaaccccgcgcgatccagttcgccgagaataccgataacaccaccagcacggtgaacatcttccatatggtatttctgggtgctcggcgcaactttacacagctgtggaaccttgcgggaaagcttatcgatatcactcatggtgaagtcgatttccgcttcctgcgccgccgccagcaggtgaagtacggtgttagtcgatccacccatcgcgatatccagcgtcatggcgttttcaaacgccgccttactggcgatattacgcggcagtgcactttcgtcgttttgctcgtaataacgtttggtcaattcaacaatgcgtttaccagcattaaggaacagctgcttacggtcggcgtgggttgccagcagcgagccgttgcccggctgcgacaggcccagcgcttcggtcaggcagttcattgagttagcggtaaacatcccggagcaggaaccgcaggtcggacacgcggaacgttcaacctgatcgctctgggagtcagatactttcgggtctgcgccctggatcatcgcatcaaccagatcgagcttgatgatctgatcggaaagtttggttttcccggcctccatcgggccgccggaaacaaagatcaccggaatattcaggcgcagggaagccatcagcatccccggggtgattttgtcgcagttagagatgcagaccatggcgtcggcgcagtgggcgttgaccatatactcaacggaatcagcgatcagttcgcgagatggcagtgaataaagcatccccccgtggcccatggcaatcccatcatccaccgcaatggtgttgaactctttggcaacgccgccagccgcttcaatttgttcggcgaccagtttaccgagatcgcgcagatggacgtgacccggtacaaattgggtgaacgagttcacaaccgcgataatcggcttaccgaaatcggcgtcggtcattccggtggcgcgccacagcgcacgagcacccgccatattacgaccatgagtggtggtggcggaacggtacttaggcatactttatttactcccagtgtctgtctcgtaaatgggacggtgcgtgccgtcccattttttgtatttcaacggatgtgctggtggaggtgatcgcctcctgatgatgagccgctcccgatgtggtgtcgggagcggtattttctataaaacttaccgcttatttgagatattcatcgaaaatgtcgagtaattcttgatgtatacacggccattcctgacctaaattgacggtacacaagccaatatcgaagccattaattttataacgatgtttcactgcggtatctacgtggggatatattaataacccccctatgttttcgccattttcaggctttaacgaccataagtaattcatcagttgataaagattttgcgaatgaaatttttctgttcccattcgtcgtgaaaaaatgctcttatagtatttggcgtcaacgataagtattttttctgatgagcgaatggtgatgtcagtttccattcgaggtaacaaattaagtgactgatccgatatactcgatgcatcccattttaaataagagcgggttgtgtttgcagacgttaattcacgacggcaaaattcataaagaaacttttgataaagtaatgacatctctttttcgtttctttcaaaatcatagaaacggtagtgtcctttgttttgacctggaatagaattattgacgatgaatttgcagacactgataacgaatttataataacgcgtattttttccgccattcagatagctgaaatgctgcggagttaaatgaagagtgctaatgcccggtaattttctataaagtgaacgagcttcatctctgatagttgaatttaacttttcatgcttaattaatatggctaatgtgctttttataattcggttagccagcgtgtcttca

SEQ ID NO: 14 - DNA, 88 bp, Artificial sequence
  source 1..88: mol_type = other DNA
tgacagctagctcagtcctaggtataatactagtgtacgcgttgccaattctatgttttagagctagaaatagcaagttaaaataagg

SEQ ID NO: 15 - DNA, 88 bp, Artificial sequence
  source 1..88: mol_type = other DNA
ccttattttaacttgctatttctagctctaaaacatagaattggcaacgcgtacactagtattatacctaggactgagctagctgtca

SEQ ID NO: 16 - DNA, 24 bp, Artificial sequence
  source 1..24: mol_type = other DNA
gtctcatgagcggatacatatttg

SEQ ID NO: 17 - DNA, 20 bp, Artificial sequence
  source 1..20: mol_type = other DNA
gcgtcaggtgcataaacaga

SEQ ID NO: 18 - DNA, 19 bp, Artificial sequence
  source 1..19: mol_type = other DNA
gagtgatgagcggttgaag

SEQ ID NO: 19 - DNA, 63 bp, Artificial sequence
  source 1..63: mol_type = other DNA
ctcacaattccacacattatacgagccggatgattaattgtcaaaaaacaggcagcaaagtcc

SEQ ID NO: 20 - DNA, 71 bp, Artificial sequence
  source 1..71: mol_type = other DNA
cgtataatgtgtggaattgtgagcggataacaatttcacacaggaaacagaccgtgcaaaaaacgcaagag

SEQ ID NO: 21 - DNA, 45 bp, Artificial sequence
  source 1..45: mol_type = other DNA
cttcacaggtagtgcttttagttagaaaagattcaccagtccaac

SEQ ID NO: 22 - DNA, 37 bp, Artificial sequence
  source 1..37: mol_type = other DNA
gtgaatcttttctaactaaaagcactacctgtgaagg

SEQ ID NO: 23 - DNA, 18 bp, Artificial sequence
  source 1..18: mol_type = other DNA
ctgcggcaataatcaacg

SEQ ID NO: 24 - DNA, 18 bp, Artificial sequence
  source 1..18: mol_type = other DNA
gcagtggcggttttcatg

SEQ ID NO: 25 - DNA, 20 bp, Artificial sequence
  source 1..20: mol_type = other DNA
ccttggtgatctcgcctttc

SEQ ID NO: 26 - DNA, 21 bp, Artificial sequence
  source 1..21: mol_type = other DNA
gctgtattccttatgtggacc

SEQ ID NO: 27 - DNA, 19 bp, Artificial sequence
  source 1..19: mol_type = other DNA
gcaggaatccaaagtcagc

SEQ ID NO: 28 - DNA, 88 bp, Artificial sequence
  source 1..88: mol_type = other DNA
tgacagctagctcagtcctaggtataatactagtctattgatattatcaatacagttttagagctagaaatagcaagttaaaataagg

SEQ ID NO: 29 - DNA, 88 bp, Artificial sequence
  source 1..88: mol_type = other DNA
ccttattttaacttgctatttctagctctaaaactgtattgataatatcaatagactagtattatacctaggactgagctagctgtca

SEQ ID NO: 30 - DNA, 18 bp, Artificial sequence
  source 1..18: mol_type = other DNA
tgaatggactgctatgcg

SEQ ID NO: 31 - DNA, 44 bp, Artificial sequence
  source 1..44: mol_type = other DNA
cacagtgtattaagcagacgttaacaacgcagtacttcctgctg

SEQ ID NO: 32 - DNA, 38 bp, Artificial sequence
  source 1..38: mol_type = other DNA
gaagtactgcgttgttaacgtctgcttaatacactgtg

SEQ ID NO: 33 - DNA, 76 bp, Artificial sequence
  source 1..76: mol_type = other DNA
gtataatgtgtggaattgtgagcggataacaatttcacacaggaaacagaccatggaactttttaaatatatggag

SEQ ID NO: 34 - DNA, 67 bp, Artificial sequence
  source 1..67: mol_type = other DNA
ctcacaattccacacattatacgagccggatgattaattgtcaattaaccccccagtttcgatttat

SEQ ID NO: 35 - DNA, 36 bp, Artificial sequence
  source 1..36: mol_type = other DNA
ccaccagcacatccgttgaaatacaaaaaatgggac

SEQ ID NO: 36 - DNA, 35 bp, Artificial sequence
  source 1..35: mol_type = other DNA
tcccattttttgtatttcaacggatgtgctggtgg

SEQ ID NO: 37 - DNA, 19 bp, Artificial sequence
  source 1..19: mol_type = other DNA
tgaagacacgctggctaac

SEQ ID NO: 38 - DNA, 18 bp, Artificial sequence
  source 1..18: mol_type = other DNA
agcgagtttccaataccg

SEQ ID NO: 39 - DNA, 18 bp, Artificial sequence
  source 1..18: mol_type = other DNA
atttctcctgctttcggc

SEQ ID NO: 40 - DNA, 88 bp, Artificial sequence
  source 1..88: mol_type = other DNA
tgacagctagctcagtcctaggtataatactagtcgtgagttaaaaaatgaactgttttagagctagaaatagcaagttaaaataagg

SEQ ID NO: 41 - DNA, 88 bp, Artificial sequence
  source 1..88: mol_type = other DNA
ccttattttaacttgctatttctagctctaaaacagttcattttttaactcacgactagtattatacctaggactgagctagctgtca

SEQ ID NO: 42 - DNA, 20 bp, Artificial sequence
  source 1..20: mol_type = other DNA
ccaatctggtgaagagcaag

SEQ ID NO: 43 - DNA, 92 bp, Artificial sequence
  source 1..92: mol_type = other DNA
ctgtttcctgtgtgaaattgttatccgctcacaattccacacattatacgagccggatgattaattgtcaatgctgaatagggtgattgttg

SEQ ID NO: 44 - DNA, 77 bp, Artificial sequence
  source 1..77: mol_type = other DNA
caatttcacacaggaaacagaccatgcgccggatattatcagtcttactcgaaaatgaatcagacgcgttattccgc

SEQ ID NO: 45 - DNA, 39 bp, Artificial sequence
  source 1..39: mol_type = other DNA
gtcttatcatgcctaccaaatcaacgcattattttatcg

SEQ ID NO: 46 - DNA, 39 bp, Artificial sequence
  source 1..39: mol_type = other DNA
cgataaaataatgcgttgatttggtaggcatgataagac

SEQ ID NO: 47 - DNA, 19 bp, Artificial sequence
  source 1..19: mol_type = other DNA
gtgcgtcctaaatcgctac

SEQ ID NO: 48 - DNA, 19 bp, Artificial sequence
  source 1..19: mol_type = other DNA
catcggcgaagagtatgag

SEQ ID NO: 49 - DNA, 20 bp, Artificial sequence
  source 1..20: mol_type = other DNA
aaagtccgaccacaccagag

SEQ ID NO: 50 - DNA, 88 bp, Artificial sequence
  source 1..88: mol_type = other DNA
tgacagctagctcagtcctaggtataatactagttcactgcccgctttccagtcgttttagagctagaaatagcaagttaaaataagg

SEQ ID NO: 51 - DNA, 88 bp, Artificial sequence
  source 1..88: mol_type = other DNA
ccttattttaacttgctatttctagctctaaaacgactggaaagcgggcagtgaactagtattatacctaggactgagctagctgtca

SEQ ID NO: 52 - DNA, 20 bp, Artificial sequence
  source 1..20: mol_type = other DNA
cggtaataatccacagcagg

SEQ ID NO: 53 - DNA, 36 bp, Artificial sequence
  source 1..36: mol_type = other DNA
gacttcgcgttcgcgtaacaggtagcagagcgggta

SEQ ID NO: 54 - DNA, 36 bp, Artificial sequence
  source 1..36: mol_type = other DNA
tacccgctctgctacctgttacgcgaacgcgaagtc

SEQ ID NO: 55 - DNA, 43 bp, Artificial sequence
  source 1..43: mol_type = other DNA
ctaactacagaaggccctacaccatgaacacgattaacatcgc

SEQ ID NO: 56 - DNA, 43 bp, Artificial sequence
  source 1..43: mol_type = other DNA
gcgatgttaatcgtgttcatggtgtagggccttctgtagttag

SEQ ID NO: 57 - DNA, 41 bp, Artificial sequence
  source 1..41: mol_type = other DNA
cattaagttctgtctcggcggagataattcacaagtgtgcg

SEQ ID NO: 58 - DNA, 41 bp, Artificial sequence
  source 1..41: mol_type = other DNA
cgcacacttgtgaattatctccgccgagacagaacttaatg

SEQ ID NO: 59 - DNA, 20 bp, Artificial sequence
  source 1..20: mol_type = other DNA
ggttacggacagaactaccg

SEQ ID NO: 60 - DNA, 18 bp, Artificial sequence
  source 1..18: mol_type = other DNA
ttcgcccattgtcgttac

SEQ ID NO: 61 - DNA, 20 bp, Artificial sequence
  source 1..20: mol_type = other DNA
agttccgcttacagcctacc

SEQ ID NO: 62 - DNA, 88 bp, Artificial sequence
  source 1..88: mol_type = other DNA
tgacagctagctcagtcctaggtataatactagtcccgtcctgcgccccgaagcgttttagagctagaaatagcaagttaaaataagg

SEQ ID NO: 63 - DNA, 88 bp, Artificial sequence
  source 1..88: mol_type = other DNA
ccttattttaacttgctatttctagctctaaaacgcttcggggcgcaggacgggactagtattatacctaggactgagctagctgtca

SEQ ID NO: 64 - DNA, 19 bp, Artificial sequence
  source 1..19: mol_type = other DNA
aaatggagggataacagcc

SEQ ID NO: 65 - DNA, 45 bp, Artificial sequence
  source 1..45: mol_type = other DNA
gctgttgcgggttaacgctccatttagaatagagtcggacgaaat

SEQ ID NO: 66 - DNA, 32 bp, Artificial sequence
  source 1..32: mol_type = other DNA
ctaaatggagcgttaacccgcaacagcaatac

SEQ ID NO: 67 - DNA, 62 bp, Artificial sequence
  source 1..62: mol_type = other DNA
gccatttacgccaagtttttgacaattaatcatccggctcgtataatgtgtggaattgtgag

SEQ ID NO: 68 - DNA, 76 bp, Artificial sequence
  source 1..76: mol_type = other DNA
cagtgtattgaagtagttagccatggtctgtttcctgtgtgaaattgttatccgctcacaattccacacattatac

SEQ ID NO: 69 - DNA, 19 bp, Artificial sequence
  source 1..19: mol_type = other DNA
ttgccttcgggcttatctc

SEQ ID NO: 70 - DNA, 20 bp, Artificial sequence
  source 1..20: mol_type = other DNA
aagacctctggaagcgtatc

SEQ ID NO: 71 - DNA, 18 bp, Artificial sequence
  source 1..18: mol_type = other DNA
cgttgcggaagtgaaatc

SEQ ID NO: 72 - DNA, 20 bp, Artificial sequence
  source 1..20: mol_type = other DNA
agttcgccctttgctctctc

SEQ ID NO: 73 - DNA, 20 bp, Artificial sequence
  source 1..20: mol_type = other DNA
agcgtttcactcctactggg